European Patent Application EP 4 151 084 A1, published March 22, 2023. Title: TRANSFECTION OF PROTOPLASTS FROM GRAPEVINE PLANTS WITH THE Cas9/gRNA COMPLEX AND REGENERATION OF RELATIVE EDITED GRAPEVINE PLANTS. Applicant: EdiVite S.r.l. The sequence listing filed with the application follows.

SEQUENCE LISTING (9 sequences)

SEQ ID NO: 1 - DNA, 21 bp, synthetic construct
  misc_feature 1..21: note = Target DNA for guide RNA for GFP
  source 1..21: mol_type = other DNA
cgagggcgacgccacctacgg

SEQ ID NO: 2 - DNA, 21 bp, synthetic construct
  misc_feature 1..21: note = Target DNA for guide RNA for GFP
  source 1..21: mol_type = other DNA
tcgccgtccagctcgaccagg

SEQ ID NO: 3 - DNA, 179 bp, Vitis vinifera
  source 1..179: mol_type = genomic DNA
atggtgagcaagggcgaggagctgttcaccggggtggtgcccatcctggtcgagctggacggcgacgtaaacggccacaagttcagcgtgtccggcgagggcgagggcgacgccacctacggcaagctgaccctgaagttcatctgcaccaccggcaagctgcccgtgccctggcccac

SEQ ID NO: 4 - DNA, 180 bp, Vitis vinifera
  source 1..180: mol_type = genomic DNA; note = CRISPR/Cas 9 edited
atggtgagcaagggcgaggagctgttcaccggggtggtgcccatcctggtcgagctggacggcgacgtaaacggccacaagttcagcgtgtccggcgagggcgagggcgacgccacactacggcaagctgaccctgaagttcatctgcaccaccggcaagctgcccgtgccctggcccac

SEQ ID NO: 5 - DNA, 115 bp, Vitis vinifera
  source 1..115: mol_type = genomic DNA
atggtgagcaagggcgaggagctgttcaccggggtggtgcccatcctggtcgagctggacggcgacgtaaacggccacaagttcagcgtgtccggcgagggcgagggcgacgcca

SEQ ID NO: 6 - DNA, 116 bp, Vitis vinifera
  source 1..116: mol_type = genomic DNA; note = CRISPR/cas 9 edited
atggtgagcaagggcgaggagctgttcaccggggtggtgcccatcctggttcgagctggacggcgacgtaaacggccacaagttcagcgtgtccggcgagggcgagggcgacgcca

SEQ ID NO: 7 - DNA, 21 bp, synthetic construct
  source 1..21: mol_type = other DNA; note = Target DNA for guide RNA for MLO17
ggagttgatggatcccatagg

SEQ ID NO: 8 - DNA, 16 bp, Vitis vinifera
  source 1..16: mol_type = genomic DNA
cctatgggatccatca

SEQ ID NO: 9 - DNA, 14 bp, Vitis vinifera
  source 1..14: mol_type = genomic DNA; note = CRISPR/Cas9 edited
cctatgaggatcca